European Patent Specification EP 3 912 642 B1, published April 12, 2023. Title: Modified antibody, antibody-conjugate and process for the preparation thereof. Applicant: SynAffix B.V. The sequence listing filed with the application follows.

SEQUENCE LISTING (24 sequences)

SEQ ID NO: 1 - DNA, 39 bp, artificial
  primer sequence
cagcgacatatgtcgctgaccgcatgccctgaggagtcc

SEQ ID NO: 2 - DNA, 36 bp, artificial
  primer sequence
gacacctccaaagttctgcacgtaaggtaggctaaa

SEQ ID NO: 3 - DNA, 39 bp, artificial
  primer sequence
ctgatggatggatccctagctcggcgtcccgatgtccac

SEQ ID NO: 4 - DNA, 36 bp, artificial
  primer sequence
ccttacgtgcagaactttggaggtgtctctgctcta

SEQ ID NO: 5 - DNA, 36 bp, artificial
  primer sequence
gacacctccaaaaaactgcacgtaaggtaggctaaa

SEQ ID NO: 6 - DNA, 36 bp, artificial
  primer sequence
ccttacgtgcagttttttggaggtgtctctgctcta

SEQ ID NO: 7 - DNA, 36 bp, artificial
  primer sequence
gacacctccaaacatctgcacgtaaggtaggctaaa

SEQ ID NO: 8 - DNA, 36 bp, artificial
  primer sequence
ccttacgtgcagatgtttggaggtgtctctgctcta

SEQ ID NO: 9 - DNA, 36 bp, artificial
  primer sequence
gacacctccaaaaatctgcacgtaaggtaggctaaa

SEQ ID NO: 10 - DNA, 36 bp, artificial
  primer sequence
ccttacgtgcagatttttggaggtgtctctgctcta

SEQ ID NO: 11 - DNA, 36 bp, artificial
  primer sequence
gacacctccaaacacctgcacgtaaggtaggctaaa

SEQ ID NO: 12 - DNA, 36 bp, artificial
  primer sequence
ccttacgtgcaggtgtttggaggtgtctctgctcta

SEQ ID NO: 13 - DNA, 36 bp, artificial
  primer sequence
gacacctccaaacgcctgcacgtaaggtaggctaaa

SEQ ID NO: 14 - DNA, 36 bp, artificial
  primer sequence
ccttacgtgcaggcgtttggaggtgtctctgctcta

SEQ ID NO: 15 - DNA, 36 bp, artificial
  primer sequence
gacacctccaaagccctgcacgtaaggtaggctaaa

SEQ ID NO: 16 - DNA, 36 bp, artificial
  primer sequence
ccttacgtgcagggctttggaggtgtctctgctcta

SEQ ID NO: 17 - protein, 402 aa, Bos taurus
MKFREPLLGGSAAMPGASLQRACRLLVAVCALHLGVTLVYYLAGRDLRRLPQLVGVHPPLQGSSHGAAAIGQPSGELRLRGVAPPPPLQNSSKPRSRAPSNLDAYSHPGPGPGPGSNLTSAPVPSTTTRSLTACPEESPLLVGPMLIEFNIPVDLKLIEQQNPKVKLGGRYTPMDCISPHKVAIIILFRNRQEHLKYWLYYLHPMVQRQQLDYGIYVINQAGESMFNRAKLLNVGFKEALKDYDYNCFVFSDVDLIPMNDHNTYRCFSQPRHISVAMDKFGFSLPYVQYFGGVSALSKQQFLSINGFPNNYWGWGGEDDDIYNRLAFRGMSVSRPNAVIGKCRMIRHSRDKKNEPNPQRFDRIAHTKETMLSDGLNSLTYMVLEVQRYPLYTKITVDIGTPS

SEQ ID NO: 18 - protein, 402 aa, artificial
  bos taurus GalT Y289N
MKFREPLLGGSAAMPGASLQRACRLLVAVCALHLGVTLVYYLAGRDLRRLPQLVGVHPPLQGSSHGAAAIGQPSGELRLRGVAPPPPLQNSSKPRSRAPSNLDAYSHPGPGPGPGSNLTSAPVPSTTTRSLTACPEESPLLVGPMLIEFNIPVDLKLIEQQNPKVKLGGRYTPMDCISPHKVAIIILFRNRQEHLKYWLYYLHPMVQRQQLDYGIYVINQAGESMFNRAKLLNVGFKEALKDYDYNCFVFSDVDLIPMNDHNTYRCFSQPRHISVAMDKFGFSLPYVQNFGGVSALSKQQFLSINGFPNNYWGWGGEDDDIYNRLAFRGMSVSRPNAVIGKCRMIRHSRDKKNEPNPQRFDRIAHTKETMLSDGLNSLTYMVLEVQRYPLYTKITVDIGTPS

SEQ ID NO: 19 - protein, 402 aa, artificial
  bos taurus GalT Y289F
MKFREPLLGGSAAMPGASLQRACRLLVAVCALHLGVTLVYYLAGRDLRRLPQLVGVHPPLQGSSHGAAAIGQPSGELRLRGVAPPPPLQNSSKPRSRAPSNLDAYSHPGPGPGPGSNLTSAPVPSTTTRSLTACPEESPLLVGPMLIEFNIPVDLKLIEQQNPKVKLGGRYTPMDCISPHKVAIIILFRNRQEHLKYWLYYLHPMVQRQQLDYGIYVINQAGESMFNRAKLLNVGFKEALKDYDYNCFVFSDVDLIPMNDHNTYRCFSQPRHISVAMDKFGFSLPYVQFFGGVSALSKQQFLSINGFPNNYWGWGGEDDDIYNRLAFRGMSVSRPNAVIGKCRMIRHSRDKKNEPNPQRFDRIAHTKETMLSDGLNSLTYMVLEVQRYPLYTKITVDIGTPS

SEQ ID NO: 20 - protein, 402 aa, artificial
  bos taurus GalT Y289M
MKFREPLLGGSAAMPGASLQRACRLLVAVCALHLGVTLVYYLAGRDLRRLPQLVGVHPPLQGSSHGAAAIGQPSGELRLRGVAPPPPLQNSSKPRSRAPSNLDAYSHPGPGPGPGSNLTSAPVPSTTTRSLTACPEESPLLVGPMLIEFNIPVDLKLIEQQNPKVKLGGRYTPMDCISPHKVAIIILFRNRQEHLKYWLYYLHPMVQRQQLDYGIYVINQAGESMFNRAKLLNVGFKEALKDYDYNCFVFSDVDLIPMNDHNTYRCFSQPRHISVAMDKFGFSLPYVQMFGGVSALSKQQFLSINGFPNNYWGWGGEDDDIYNRLAFRGMSVSRPNAVIGKCRMIRHSRDKKNEPNPQRFDRIAHTKETMLSDGLNSLTYMVLEVQRYPLYTKITVDIGTPS

SEQ ID NO: 21 - protein, 402 aa, artificial
  bos taurus GalT Y289I
MKFREPLLGGSAAMPGASLQRACRLLVAVCALHLGVTLVYYLAGRDLRRLPQLVGVHPPLQGSSHGAAAIGQPSGELRLRGVAPPPPLQNSSKPRSRAPSNLDAYSHPGPGPGPGSNLTSAPVPSTTTRSLTACPEESPLLVGPMLIEFNIPVDLKLIEQQNPKVKLGGRYTPMDCISPHKVAIIILFRNRQEHLKYWLYYLHPMVQRQQLDYGIYVINQAGESMFNRAKLLNVGFKEALKDYDYNCFVFSDVDLIPMNDHNTYRCFSQPRHISVAMDKFGFSLPYVQIFGGVSALSKQQFLSINGFPNNYWGWGGEDDDIYNRLAFRGMSVSRPNAVIGKCRMIRHSRDKKNEPNPQRFDRIAHTKETMLSDGLNSLTYMVLEVQRYPLYTKITVDIGTPS

SEQ ID NO: 22 - protein, 402 aa, artificial
  bos taurus GalT Y289V
MKFREPLLGGSAAMPGASLQRACRLLVAVCALHLGVTLVYYLAGRDLRRLPQLVGVHPPLQGSSHGAAAIGQPSGELRLRGVAPPPPLQNSSKPRSRAPSNLDAYSHPGPGPGPGSNLTSAPVPSTTTRSLTACPEESPLLVGPMLIEFNIPVDLKLIEQQNPKVKLGGRYTPMDCISPHKVAIIILFRNRQEHLKYWLYYLHPMVQRQQLDYGIYVINQAGESMFNRAKLLNVGFKEALKDYDYNCFVFSDVDLIPMNDHNTYRCFSQPRHISVAMDKFGFSLPYVQVFGGVSALSKQQFLSINGFPNNYWGWGGEDDDIYNRLAFRGMSVSRPNAVIGKCRMIRHSRDKKNEPNPQRFDRIAHTKETMLSDGLNSLTYMVLEVQRYPLYTKITVDIGTPS

SEQ ID NO: 23 - protein, 402 aa, artificial
  bos taurus GalT Y289A
MKFREPLLGGSAAMPGASLQRACRLLVAVCALHLGVTLVYYLAGRDLRRLPQLVGVHPPLQGSSHGAAAIGQPSGELRLRGVAPPPPLQNSSKPRSRAPSNLDAYSHPGPGPGPGSNLTSAPVPSTTTRSLTACPEESPLLVGPMLIEFNIPVDLKLIEQQNPKVKLGGRYTPMDCISPHKVAIIILFRNRQEHLKYWLYYLHPMVQRQQLDYGIYVINQAGESMFNRAKLLNVGFKEALKDYDYNCFVFSDVDLIPMNDHNTYRCFSQPRHISVAMDKFGFSLPYVQAFGGVSALSKQQFLSINGFPNNYWGWGGEDDDIYNRLAFRGMSVSRPNAVIGKCRMIRHSRDKKNEPNPQRFDRIAHTKETMLSDGLNSLTYMVLEVQRYPLYTKITVDIGTPS

SEQ ID NO: 24 - protein, 402 aa, artificial
  bos taurus GalT Y289G
MKFREPLLGGSAAMPGASLQRACRLLVAVCALHLGVTLVYYLAGRDLRRLPQLVGVHPPLQGSSHGAAAIGQPSGELRLRGVAPPPPLQNSSKPRSRAPSNLDAYSHPGPGPGPGSNLTSAPVPSTTTRSLTACPEESPLLVGPMLIEFNIPVDLKLIEQQNPKVKLGGRYTPMDCISPHKVAIIILFRNRQEHLKYWLYYLHPMVQRQQLDYGIYVINQAGESMFNRAKLLNVGFKEALKDYDYNCFVFSDVDLIPMNDHNTYRCFSQPRHISVAMDKFGFSLPYVQGFGGVSALSKQQFLSINGFPNNYWGWGGEDDDIYNRLAFRGMSVSRPNAVIGKCRMIRHSRDKKNEPNPQRFDRIAHTKETMLSDGLNSLTYMVLEVQRYPLYTKITVDIGTPS